European Patent Specification EP 3 965 891 B1, published July 8, 2026. Title: ANTIBODY DRUG CONJUGATES. Applicant: TAKEDA PHARMACEUTICAL COMPANY, LTD. The sequence listing filed with the application follows.

SEQUENCE LISTING (4 sequences)

SEQ ID NO: 1 - protein, 485 aa, Artificial Sequence
  Heavy Chain
MGWSCIILFLVATATGVHSQVQLQQWGAGLLKPSETLSLTCAVFGGSFSGYYWSWIRQPPGKGLEWIGEINHRGNTNDNPSLKSRVTISVDTSKNQFALKLSSVTAADTAVYYCARERGYTYGNFDHWGQGTLVTVSSASTKGPSVFPLAPSSKSTSGGTAALGCLVKDYFPEPVTVSWNSGALTSGVHTFPAVLQSSGLYSLSSVVTVPSSSLGTQTYICNVNHKPSNTKVDKKVEPKSCDKTHTCPPCPAPELLGGPSVFLFPPKPKDTLMISRTPEVTCVVVDVSHEDPEVKFNWYVDGVEVHNAKTKPREEQYNSTYRVVSVLTVLHQDWLNGKEYKCKVSNKALPAPIEKTISKAKGQPREPQVYTLPPSRDELTKNQVSLTCLVKGFYPSDIAVEWESNGQPENNYKTTPPVLDSDGSFFLYSKLTVDKSRWQQGNVFSCSVMHEALHNHYTQKSLSLSPGKAGGGSLPETGGHHHHHH

SEQ ID NO: 2 - protein, 233 aa, Artificial Sequence
  Light Chain Sequence
MGWSCIILFLVATATGVHSEIVMTQSPATLSVSPGERATLSCRASQSVSRNLAWYQQKPGQAPRLLIYGASTRATGIPARFSGSGSGTEFTLTIGSLQSEDFAVYYCQQYKTWPRTFGQGTNVEIKRTVAAPSVFIFPPSDEQLKSGTASVVCLLNNFYPREAKVQWKVDNALQSGNSQESVTEQDSKDSTYSLSSTLTLSKADYEKHKVYACEVTHQGLSSPVTKSFNRGEC

SEQ ID NO: 3 - protein, 12 aa, Artificial Sequence
  heavy chain constant region
HHHHHHGGTPEL

SEQ ID NO: 4 - protein, 12 aa, Artificial Sequence
  heavy chain constant region
LPETGGHHHHHH